European Patent Application EP 4 610 280 A1, published September 3, 2025. Title: METHOD FOR PRODUCING POLYPEPTIDE FROM RECOMBINANT FUSION PROTEIN AND USE THEREOF. Applicant: YANGZHOU AURISCO PHARMACEUTICAL CO., LTD. The sequence listing filed with the application follows.

SEQUENCE LISTING (42 sequences)

SEQ ID NO: 1 - protein, 5 aa, synthetic construct
DDDDK

SEQ ID NO: 2 - protein, 5 aa, synthetic construct
EQIGG

SEQ ID NO: 3 - protein, 6 aa, synthetic construct
LVPRGS

SEQ ID NO: 4 - protein, 7 aa, synthetic construct
  REGION 7: note = X= G or S
ENLYFQX

SEQ ID NO: 5 - DNA, 53 bp, synthetic construct
  source 1..53: mol_type = other DNA
tgcggccgcaagcttgtcgacggagctcgaattcttattagccgcggccacga

SEQ ID NO: 6 - DNA, 37 bp, synthetic construct
  source 1..37: mol_type = other DNA
cagttttattgttcatgaccaaaatcccttaacgtga

SEQ ID NO: 7 - DNA, 41 bp, synthetic construct
  source 1..41: mol_type = other DNA
ctaagaattaattcatgagcggatacatatttgaatgtatt

SEQ ID NO: 8 - protein, 163 aa, synthetic construct
MSPIKEDPINEIDELDSILNTMAQNIIRTSYSRDKTFSNIQTKCCNTVIEGGISIRSYSEFIQLINSCRVAFVLITTTYCPYCQLFKPVFFRVAREFAGKAVFIEANADYVPEVAETFNVYSTPTTVIIIDKRPIDAILGYIPYNHFKRYVNDIVSYAECGEI

SEQ ID NO: 9 - DNA, 489 bp, synthetic construct
  source 1..489: mol_type = other DNA
atgagcccgattaaagaagatccgatcaacgaaattgatgaactggatagcattctgaacaccatggcccagaatattatccgtacctcctatagccgcgataaaacctttagcaacatccagaccaaatgctgcaacaccgtgatcgagggtggcattagcatccgcagctacagcgaatttatccagctgatcaacagctgccgcgtggcgtttgtgctgatcaccaccacctactgcccgtattgccagctgtttaaaccggtgtttttccgcgtggcccgcgaatttgccggcaaagccgttttcatcgaagccaacgccgattatgtgcccgaagtggcggaaacctttaacgtgtatagcaccccgaccacggtgatcattatcgacaaacgcccgattgatgcgattctgggctacatcccgtataaccattttaaacgctatgtgaacgatattgtgagctacgccgaatgcggcgagatt

SEQ ID NO: 10 - protein, 146 aa, synthetic construct
MTPDAWDEFDSLWDEYVAKAVEAAKRAGVVLARSYDEYRKAICSKPVAVVVFTSPTCPACAAYRPIFYEYARRMSQYRGKVAFVEVDSYSAYEAAMEAGVMATPTTVVYLKCKPVDGFIGLADEETLDEIVRPYITKAVEEGEEDE

SEQ ID NO: 11 - DNA, 438 bp, synthetic construct
  source 1..438: mol_type = other DNA
atgaccccggatgcatgggatgaatttgatagcctgtgggatgaatatgttgcaaaagcagttgaagcagcaaaacgtgcaggtgttgttctggcacgtagctatgatgaatatcgtaaagcaatttgtagcaaaccggtggcagttgttgtttttaccagcccgacctgtccggcatgtgcagcatatcgtccgattttctatgaatatgcacgtcgtatgagccagtatcgtggtaaagttgcatttgttgaagttgatagctatagcgcatatgaagcagcaatggaagcaggtgttatggcaaccccgaccaccgttgtttatctgaaatgtaaaccggttgatggttttattggtctggcagatgaagaaaccctggatgaaattgttcgtccgtatattaccaaagcagttgaagaaggtgaagaagatgaa

SEQ ID NO: 12 - protein, 147 aa, synthetic construct
MATCIVLRLHQGEGLGLLRLTSKSELDRVIRGSRFALVVFTGLACPACEMYKPVLEKLAELVGKDMPVVEYVVDYDPEPALELGIMGTPTTVVYVDGKPVEGFVGAVDLPDLLEFLAKVASKSDKQLAEKLEKLAEKVKPLYGGLYW

SEQ ID NO: 13 - DNA, 441 bp, synthetic construct
  source 1..441: mol_type = other DNA
atggcaacctgtattgttctgcgtctgcatcagggtgaaggtctgggtctgctgcgtctgaccagcaaaagcgaactggatcgtgttattcgtggtagccgttttgcactggttgtgtttaccggtctggcatgtccggcatgtgaaatgtataaaccggttctggaaaaactggcagaactggttggtaaagatatgccggttgttgaatatgttgttgattatgatccggaaccggcactggaactgggtattatgggtacaccgaccaccgttgtttatgttgatggtaaaccggttgaaggttttgttggtgcagttgatctgccggatctgctggaatttctggcaaaagttgcaagcaaaagcgataaacagctggcagaaaaactggaaaaactggccgaaaaagttaaaccgctgtatggtggtctgtattgg

SEQ ID NO: 14 - protein, 148 aa, synthetic construct
MRGWHRMSSVDEVAAELRKLVEQKIRRIEQDLGDPLYYIEKDFDKVIERYPVAVVEFSAPWCNPCKAYTPVFRRVARRLIEEYNGKVLFAYLDTDKLPETADRYNVENIPTTIIFVNGHVADVIMGATTESRLEDKVRSILKEVVGGK

SEQ ID NO: 15 - DNA, 444 bp, synthetic construct
  source 1..444: mol_type = other DNA
atgcgtggttggcatcgcatgagcagcgttgatgaagttgcagcagaactgcgtaaactggttgaacagaaaattcgtcgtattgaacaggatctgggtgatccgctgtattatattgaaaaagattttgataaagttattgaacgttatccggttgcagttgttgaatttagcgcaccgtggtgtaatccgtgtaaagcatataccccggtttttcgtcgtgttgcccgtcgtctgattgaagaatataatggtaaagttctgtttgcatatctggataccgataaactgccggaaaccgcagatcgttataatgttgaaaatattccgaccaccattatttttgttaatggtcatgttgcagatgttattatgggtgcaaccaccgaaagccgtctggaagataaagttcgtagcattctgaaagaagttgttggtggtaaa

SEQ ID NO: 16 - protein, 116 aa, synthetic construct
MLFKRREKEGNIVEIPCDSKEFKKIIEENKVVVVDFWAKWCFPCLIYARSFKKAANRLVGRALFAKVNVGECYSLARKYNIFGVPTTMIFVNGKPKRRILGPVSDKALVRIVEEYL

SEQ ID NO: 17 - DNA, 348 bp, synthetic construct
  source 1..348: mol_type = other DNA
atgctgtttaaacgccgcgaaaaagaaggcaacattgtggaaatcccgtgcgatagcaaagaatttaagaaaattatcgaagagaacaaagtggtggtggtggatttttgggcgaaatggtgctttccgtgcctgatttatgcccgcagctttaaaaaagccgccaatcgcctggtgggccgcgcgctgtttgccaaagtgaatgtgggcgaatgctatagcctggcccgcaaatacaacatttttggcgtgccgaccaccatgatctttgtgaacggcaaaccgaaacgccgcatcctgggcccggtgagcgataaagcgctggtgcgcattgtggaagaatatctg

SEQ ID NO: 18 - protein, 109 aa, synthetic construct
MSDKIIHLTDDSFDTDVLKADGAILVDFWAEWCGPCKMIAPILDEIADEYQGKLTVAKLNIDQNPGTAPKYGIRGIPTLLLFKNGEVAATKVGALSKGQLKEFLDANLA

SEQ ID NO: 19 - DNA, 327 bp, synthetic construct
  source 1..327: mol_type = other DNA
atgagcgataaaattattcacctgactgacgacagttttgacacggatgtactcaaagcggacggggcgatcctcgtcgatttctgggcagagtggtgcggtccgtgcaaaatgatcgccccgattctggatgaaatcgctgacgaatatcagggcaaactgaccgttgcaaaactgaacatcgatcaaaaccctggcactgcgccgaaatatggcatccgtggtatcccgactctgctgctgttcaaaaacggtgaagtggcggcaaccaaagtgggtgcactgtctaaaggtcagttgaaagagttcctcgacgctaacctggcc

SEQ ID NO: 20 - protein, 403 aa, synthetic construct
DDDDKEGTFTSDVSSYLEGQAAKEFIAWLVRGRGKRGSGSGDDDDKEGTFTSDVSSYLEGQAAKEFIAWLVRGRGKRGSGSGDDDDKEGTFTSDVSSYLEGQAAKEFIAWLVRGRGKRGSGSGDDDDKEGTFTSDVSSYLEGQAAKEFIAWLVRGRGKRGSGSGDDDDKEGTFTSDVSSYLEGQAAKEFIAWLVRGRGKRGSGSGDDDDKEGTFTSDVSSYLEGQAAKEFIAWLVRGRGKRGSGSGDDDDKEGTFTSDVSSYLEGQAAKEFIAWLVRGRGKRGSGSGDDDDKEGTFTSDVSSYLEGQAAKEFIAWLVRGRGKRGSGSGDDDDKEGTFTSDVSSYLEGQAAKEFIAWLVRGRGKRGSGSGDDDDKEGTFTSDVSSYLEGQAAKEFIAWLVRGRG

SEQ ID NO: 21 - DNA, 1212 bp, synthetic construct
  source 1..1212: mol_type = other DNA
gacgacgatgacaaagaaggtacgtttacgagcgacgttagcagttatctggaaggccaagcggcgaaagaatttatcgcctggctggtgcgcggtcgtggcaaacgtggcagcggtagcggcgatgacgatgacaaggagggcaccttcacgagcgacgttagcagttatttagaaggccaagccgccaaagagtttattgcgtggctggttcgcggtcgtggcaaacgtggtagtggcagcggcgacgacgacgacaaagaaggcacgttcacgagcgacgttagcagctatctggaaggccaagcggccaaagagtttattgcctggctggtgcgcggccgtggcaagcgcggcagcggcagtggtgacgatgacgataaagagggcacctttacgagcgatgtgagcagctatttagagggtcaagcggcgaaggagtttattgcgtggttagtgcgcggccgcggcaaacgcggtagcggcagtggcgacgacgacgataaggaaggcacgtttacgagcgacgtgagtagctacctggaaggtcaagccgccaaggagtttattgcgtggttagttcgtggccgtggcaaacgcggtagtggcagtggcgacgatgatgacaaagagggcaccttcacgagcgatgtgagtagctatctggaaggccaagcggccaaagaatttatcgcgtggctggtgcgtggccgtggcaaacgcggcagcggcagcggcgatgatgacgataaagagggcaccttcacgagcgatgttagtagttatctggagggccaagcggcgaaagagtttattgcctggctggtgcgtggtcgtggcaaacgtggcagtggcagtggcgatgacgatgacaaagagggcacctttacgagcgatgtgagtagctatctggaaggccaagcggcgaaagagtttatcgcctggctggtgcgcggtcgtggtaagcgcggcagcggcagtggcgatgacgacgataaggaaggcaccttcacgagcgatgtgagcagttatctggaaggccaagcggcgaaagagtttattgcgtggttagttcgcggtcgtggcaaacgcggcagcggtagcggtgatgacgatgataaagagggcacgtttacgagcgacgtgagcagctacctggagggtcaagcggccaaagaatttattgcgtggctggttcgtggccgcggctaa

SEQ ID NO: 22 - protein, 116 aa, synthetic construct
DDDDKEGTFTSDVSSYLEGQAAKEFIAWLVRGRGKRGSGSGDDDDKEGTFTSDVSSYLEGQAAKEFIAWLVRGRGKRGSGSGDDDDKEGTFTSDVSSYLEGQAAKEFIAWLVRGRG

SEQ ID NO: 23 - DNA, 372 bp, synthetic construct
  source 1..372: mol_type = other DNA
gacgacgacgataaagaaggtacttttacctccgatgtatcttcctacctggagggccaggctgctaaagaattcatcgcatggctggtgcgtggtcgtggtaagcgtggctctggctccggcgacgacgacgacaaagaaggcacgtttacctccgacgttagctcttacctggaaggtcaagctgctaaagaatttatcgcgtggctggtgcgtggccgtggtaaacgtggttccggctctggtgacgatgacgacaaagaaggcaccttcacgtctgatgtttcctcctatctggaaggccaggccgccaaagagttcatcgcgtggctggttcgtggtcgtggtaaacgtggttccggtagcggctaa

SEQ ID NO: 24 - protein, 157 aa, synthetic construct
DDDDKEGTFTSDVSSYLEGQAAKEFIAWLVRGRGKRGSGSGDDDDKEGTFTSDVSSYLEGQAAKEFIAWLVRGRGKRGSGSGDDDDKEGTFTSDVSSYLEGQAAKEFIAWLVRGRGKRGSGSGDDDDKEGTFTSDVSSYLEGQAAKEFIAWLVRGRG

SEQ ID NO: 25 - DNA, 474 bp, synthetic construct
  source 1..474: mol_type = other DNA
gacgatgacgacaaagaaggcaccttcacgagcgatgttagcagttatctggaaggtcaagccgccaaagagttcattgcctggttagttcgcggccgcggcaaacgcggtagtggcagcggcgacgatgatgacaaagaaggcaccttcacgagcgatgtgagcagctatctggaaggccaagcggcgaaggagtttatcgcgtggctggttcgcggccgcggcaaacgcggcagcggcagtggcgatgacgatgataaggagggcacgtttacgagcgatgtgagcagttacctggaaggccaagcggcgaaggagttcattgcgtggctggtgcgtggccgtggtaagcgtggcagcggtagcggcgacgatgatgacaaagagggcaccttcacgagtgacgttagtagctatttagaaggccaagcggccaaagaatttatcgcctggttagtgcgcggtcgtggctaa

SEQ ID NO: 26 - protein, 198 aa, synthetic construct
DDDDKEGTFTSDVSSYLEGQAAKEFIAWLVRGRGKRGSGSGDDDDKEGTFTSDVSSYLEGQAAKEFIAWLVRGRGKRGSGSGDDDDKEGTFTSDVSSYLEGQAAKEFIAWLVRGRGKRGSGSGDDDDKEGTFTSDVSSYLEGQAAKEFIAWLVRGRGKRGSGSGDDDDKEGTFTSDVSSYLEGQAAKEFIAWLVRGRG

SEQ ID NO: 27 - DNA, 597 bp, synthetic construct
  source 1..597: mol_type = other DNA
gacgatgatgacaaagaaggcacctttacgagcgacgtgagcagttacctggaaggccaagccgcgaaagagtttattgcctggctggtgcgcggccgtggcaaacgtggcagtggcagcggcgacgatgacgacaaggagggcacctttacgagcgacgttagcagctacttagaaggccaagcggccaaggaatttatcgcctggctggtgcgcggtcgcggcaaacgcggtagcggcagtggtgatgacgatgacaaggaaggcaccttcacgagcgatgtgagtagttatctggaaggccaagccgcgaaggaatttatcgcgtggttagttcgcggccgtggtaaacgcggcagcggcagcggcgacgatgacgataaggaaggcaccttcacgagcgacgttagcagctacctggaaggccaagcggccaaagagttcatcgcgtggctggtgcgtggtcgcggtaaacgcggtagtggcagcggcgatgacgatgataaggagggcaccttcacgagcgatgttagtagttacctggaaggtcaagcggcgaaagaatttattgcctggttagtgcgtggccgcggttaa

SEQ ID NO: 28 - protein, 239 aa, synthetic construct
DDDDKEGTFTSDVSSYLEGQAAKEFIAWLVRGRGKRGSGSGDDDDKEGTFTSDVSSYLEGQAAKEFIAWLVRGRGKRGSGSGDDDDKEGTFTSDVSSYLEGQAAKEFIAWLVRGRGKRGSGSGDDDDKEGTFTSDVSSYLEGQAAKEFIAWLVRGRGKRGSGSGDDDDKEGTFTSDVSSYLEGQAAKEFIAWLVRGRGKRGSGSGDDDDKEGTFTSDVSSYLEGQAAKEFIAWLVRGRG

SEQ ID NO: 29 - DNA, 720 bp, synthetic construct
  source 1..720: mol_type = other DNA
gatgatgacgataaagagggcaccttcacgagcgacgttagtagttacttagagggtcaagcggcgaaggaatttattgcctggttagttcgcggccgtggtaagcgtggtagtggcagtggcgacgatgacgataaagaaggtacgttcacgagtgacgttagtagctacctggagggccaagcggccaaagagttcatcgcctggctggttcgcggtcgtggcaagcgcggcagcggcagcggcgatgacgatgataaagaaggcacctttacgagcgacgtgagcagctatctggagggtcaagcggcgaaagaatttatcgcgtggctggttcgcggccgtggtaaacgtggcagcggcagcggtgacgacgacgataaagaaggcacgttcacgagcgatgtgagcagttatttagaaggccaagcggcgaaggagtttatcgcgtggctggtgcgtggtcgtggcaaacgcggcagcggtagtggcgatgatgacgacaaagaaggcacgtttacgagtgatgtgagtagttatttagagggtcaagcggcgaaagagttcatcgcgtggctggtgcgcggccgcggtaaacgtggcagcggcagtggcgatgacgatgataaagagggcacctttacgagcgatgtgagcagctatttagaaggccaagcggcgaaagaatttattgcgtggctggttcgcggtcgtggctaa

SEQ ID NO: 30 - DNA, 42 bp, synthetic construct
  source 1..42: mol_type = other DNA
atccgctcatgaattaattcttagaaaaactcatcgagcatc

SEQ ID NO: 31 - DNA, 42 bp, synthetic construct
  source 1..42: mol_type = other DNA
attttggtcatgaacaataaaactgtctgcttacataaacag

SEQ ID NO: 32 - DNA, 64 bp, synthetic construct
  source 1..64: mol_type = other DNA
gctctagaaataattttgtttaactttaagaaggagatatacatatgagcccgattaaagaaga

SEQ ID NO: 33 - DNA, 28 bp, synthetic construct
  source 1..28: mol_type = other DNA
ggggtaccaatctcgccgcattcggcgt

SEQ ID NO: 34 - DNA, 64 bp, synthetic construct
  source 1..64: mol_type = other DNA
gctctagaaataattttgtttaactttaagaaggagatatacatatgaccccggatgcatggga

SEQ ID NO: 35 - DNA, 29 bp, synthetic construct
  source 1..29: mol_type = other DNA
ggggtaccttcatcttcttcaccttcttc

SEQ ID NO: 36 - DNA, 64 bp, synthetic construct
  source 1..64: mol_type = other DNA
gctctagaaataattttgtttaactttaagaaggagatatacatatggcaacctgtattgttct

SEQ ID NO: 37 - DNA, 29 bp, synthetic construct
  source 1..29: mol_type = other DNA
ggggtaccccaatacagaccaccatacag

SEQ ID NO: 38 - DNA, 64 bp, synthetic construct
  source 1..64: mol_type = other DNA
gctctagaaataattttgtttaactttaagaaggagatatacatatgcgtggttggcatcgcat

SEQ ID NO: 39 - DNA, 29 bp, synthetic construct
  source 1..29: mol_type = other DNA
ggggtacctttaccaccaacaacttcttt

SEQ ID NO: 40 - DNA, 64 bp, synthetic construct
  source 1..64: mol_type = other DNA
gctctagaaataattttgtttaactttaagaaggagatatacatatgctgtttaaacgccgcga

SEQ ID NO: 41 - DNA, 29 bp, synthetic construct
  source 1..29: mol_type = other DNA
ggggtacccagatattcttccacaatgcg

SEQ ID NO: 42 - DNA, 79 bp, synthetic construct
  source 1..79: mol_type = other DNA
ataacaattcccctctagaaataattttgtttaactttaagaaggagatatacatatgggtaccgacgacgatgacaaa